European Patent Specification EP 3 456 737 B1, published February 14, 2024. Title: Antibody variants. Applicant: Tillotts Pharma AG. The sequence listing filed with the application follows.

SEQUENCE LISTING (24 sequences)

SEQ ID NO: 1 - protein, 221 aa, Artificial Sequence
  Light chain of Ab-wt, the parent antibody of the modified antibodies used in the examples (clone 16-22-H05)
DIQMTQSPSSLSASVGDRVTIKCQASQSIFSGLAWYQQKPGKAPKLLIYGASKLASGVPSRFSGSGSGTEFTLTISGLQPADFATYYCQSYYYSSSSSDGSYAFGGGTKLTVLGRTVAAPSVFIFPPSDEQLKSGTASVVCLLNNFYPREAKVQWKVDNALQSGNSQESVTEQDSKDSTYSLSSTLTLSKADYEKHKVYACEVTHQGLSSPVTKSFNRGEC

SEQ ID NO: 2 - protein, 452 aa, Artificial Sequence
  Heavy chain of Ab-wt, the parent antibody of the modified antibodies used in the examples (clone 16-22-H05)
EVQLVESGGGLVQPGGSLRLSCKASGIDFNNYGIGWVRQAPGKGLEWITYIYPGFAITNFANSVKGRFTISSDNSKNTVYLQMNSLRAEDTAVYYCARDPVYATSSGYFDLWGQGTLVTVSSASTKGPSVFPLAPSSKSTSGGTAALGCLVKDYFPEPVTVSWNSGALTSGVHTFPAVLQSSGLYSLSSVVTVPSSSLGTQTYICNVNHKPSNTKVDKKVEPKSCDKTHTCPPCPAPELLGGPSVFLFPPKPKDTLMISRTPEVTCVVVDVSHEDPEVKFNWYVDGVEVHNAKTKPREEQYNSTYRVVSVLTVLHQDWLNGKEYKCKVSNKALPAPIEKTISKAKGQPREPQVYTLPPSREEMTKNQVSLTCLVKGFYPSDIAVEWESNGQPENNYKTTPPVLDSDGSFFLYSKLTVDKSRWQQGNVFSCSVMHEALHNHYTQKSLSLSPGK

SEQ ID NO: 3 - protein, 11 aa, Artificial Sequence
  CDR L1 of clone 16-22-H05
QASQSIFSGLA

SEQ ID NO: 4 - protein, 7 aa, Artificial Sequence
  CDR L2 of clone 16-22-H05
GASKLAS

SEQ ID NO: 5 - protein, 15 aa, Artificial Sequence
  CDR L3 of clone 16-22-H05
QSYYYSSSSSDGSYA

SEQ ID NO: 6 - protein, 10 aa, Artificial Sequence
  CDR H1 of clone 16-22-H05
GIDFNNYGIG

SEQ ID NO: 7 - protein, 17 aa, Artificial Sequence
  CDR H2 of clone 16-22-H05
YIYPGFAITNFANSVKG

SEQ ID NO: 8 - protein, 13 aa, Artificial Sequence
  CDR H3 of clone 16-22-H05
DPVYATSSGYFDL

SEQ ID NO: 9 - protein, 122 aa, Artificial Sequence
  VH of humanized IgG of clone 16-22-H05
EVQLVESGGGLVQPGGSLRLSCKASGIDFNNYGIGWVRQAPGKGLEWITYIYPGFAITNFANSVKGRFTISSDNSKNTVYLQMNSLRAEDTAVYYCARDPVYATSSGYFDLWGQGTLVTVSS

SEQ ID NO: 10 - protein, 114 aa, Artificial Sequence
  VL of humanized IgG of clone 16-22-H05
DIQMTQSPSSLSASVGDRVTIKCQASQSIFSGLAWYQQKPGKAPKLLIYGASKLASGVPSRFSGSGSGTEFTLTISGLQPADFATYYCQSYYYSSSSSDGSYAFGGGTKLTVLG

SEQ ID NO: 11 - protein, 452 aa, Artificial Sequence
  Heavy chain of Ab-AA (based on clone 16-22-H05)
EVQLVESGGGLVQPGGSLRLSCKASGIDFNNYGIGWVRQAPGKGLEWITYIYPGFAITNFANSVKGRFTISSDNSKNTVYLQMNSLRAEDTAVYYCARDPVYATSSGYFDLWGQGTLVTVSSASTKGPSVFPLAPSSKSTSGGTAALGCLVKDYFPEPVTVSWNSGALTSGVHTFPAVLQSSGLYSLSSVVTVPSSSLGTQTYICNVNHKPSNTKVDKKVEPKSCDKTHTCPPCPAPELLGGPSVFLFPPKPKDTLMISRTPEVTCVVVDVSHEDPEVKFNWYVDGVEVHNAKTKPREEQYNSTYRVVSVLTVLHQDWLNGKEYKCKVSNKALPAPIEKTISKAKGQPREPQVYTLPPSREEMTKNQVSLTCLVKGFYPSDIAVAWESNGQPENNYKTTPPVLDSDGSFFLYSKLTVDKSRWQQGNVFSCSVMHEALHAHYTQKSLSLSPGK

SEQ ID NO: 12 - protein, 454 aa, Artificial Sequence
  Heavy chain of Ab-AA (based on clone 17-22-B03)
EVQLVESGGGLVQPGGSLRLSCKASGIDFSAGYDMCWVRQAPGKGLEWIACIDSRREESDYASWAKGRFTISKDSSKNTVYLQMNSLRAEDTAVYYCARGGYGGDGVDGAFDPWGQGTLVTVSSASTKGPSVFPLAPSSKSTSGGTAALGCLVKDYFPEPVTVSWNSGALTSGVHTFPAVLQSSGLYSLSSVVTVPSSSLGTQTYICNVNHKPSNTKVDKKVEPKSCDKTHTCPPCPAPELLGGPSVFLFPPKPKDTLMISRTPEVTCVVVDVSHEDPEVKFNWYVDGVEVHNAKTKPREEQYNSTYRVVSVLTVLHQDWLNGKEYKCKVSNKALPAPIEKTISKAKGQPREPQVYTLPPSREEMTKNQVSLTCLVKGFYPSDIAVAWESNGQPENNYKTTPPVLDSDGSFFLYSKLTVDKSRWQQGNVFSCSVMHEALHAHYTQKSLSLSPGK

SEQ ID NO: 13 - protein, 232 aa, Artificial Sequence
  Fc region of Ab-AA (including hinge region)
EPKSCDKTHTCPPCPAPELLGGPSVFLFPPKPKDTLMISRTPEVTCVVVDVSHEDPEVKFNWYVDGVEVHNAKTKPREEQYNSTYRVVSVLTVLHQDWLNGKEYKCKVSNKALPAPIEKTISKAKGQPREPQVYTLPPSREEMTKNQVSLTCLVKGFYPSDIAVAWESNGQPENNYKTTPPVLDSDGSFFLYSKLTVDKSRWQQGNVFSCSVMHEALHAHYTQKSLSLSPGK

SEQ ID NO: 14 - protein, 11 aa, Artificial Sequence
  CDR L1 of clone 17-22-B03
QASQSISSYLA

SEQ ID NO: 15 - protein, 7 aa, Artificial Sequence
  CDR L2 of clone 17-22-B03
KASTLAS

SEQ ID NO: 16 - protein, 13 aa, Artificial Sequence
  CDR L3 of clone 17-22-B03
QCTYYEPSYVFRA

SEQ ID NO: 17 - protein, 11 aa, Artificial Sequence
  CDR H1 of clone 17-22-B03
GIDFSAGYDMC

SEQ ID NO: 18 - protein, 17 aa, Artificial Sequence
  CDR H2 of clone 17-22-B03
CIDSRREESDYASWAKG

SEQ ID NO: 19 - protein, 14 aa, Artificial Sequence
  CDR H3 of clone 17-22-B03
GGYGGDGVDGAFDP

SEQ ID NO: 20 - protein, 124 aa, Artificial Sequence
  VH of humanized IgG of clone 17-22-B03
EVQLVESGGGLVQPGGSLRLSCKASGIDFSAGYDMCWVRQAPGKGLEWIACIDSRREESDYASWAKGRFTISKDSSKNTVYLQMNSLRAEDTAVYYCARGGYGGDGVDGAFDPWGQGTLVTVSS

SEQ ID NO: 21 - protein, 112 aa, Artificial Sequence
  VL of humanized IgG of clone 17-22-B03 -(sc08)
DIQMTQSPSSLSASVGDRVTITCQASQSISSYLAWYQQKPGKAPKLLIYKASTLASGVPSRFSGSGSGTDFTLTISSLQPEDFATYYCQCTYYEPSYVFRAFGGGTKLTVLG

SEQ ID NO: 22 - protein, 112 aa, Artificial Sequence
  VL of humanized IgG of clone 17-22-B03 -(sc02)
DIQMTQSPSSLSASVGDRVTIKCQASQSISSYLAWYQQKPGKAPKLLIYKASTLASGVPSRFSGSGSGTEFTLTISDLEPADFATYYCQCTYYEPSYVFRAFGGGTKLTVLG

SEQ ID NO: 23 - protein, 219 aa, Artificial Sequence
  Light chain of humanized IgG of clone 17-22-B03 -(sc08)
DIQMTQSPSSLSASVGDRVTITCQASQSISSYLAWYQQKPGKAPKLLIYKASTLASGVPSRFSGSGSGTDFTLTISSLQPEDFATYYCQCTYYEPSYVFRAFGGGTKLTVLGRTVAAPSVFIFPPSDEQLKSGTASVVCLLNNFYPREAKVQWKVDNALQSGNSQESVTEQDSKDSTYSLSSTLTLSKADYEKHKVYACEVTHQGLSSPVTKSFNRGEC

SEQ ID NO: 24 - protein, 219 aa, Artificial Sequence
  Light chain of humanized IgG of clone 17-22-B03 -(sc02)
DIQMTQSPSSLSASVGDRVTIKCQASQSISSYLAWYQQKPGKAPKLLIYKASTLASGVPSRFSGSGSGTEFTLTISDLEPADFATYYCQCTYYEPSYVFRAFGGGTKLTVLGRTVAAPSVFIFPPSDEQLKSGTASVVCLLNNFYPREAKVQWKVDNALQSGNSQESVTEQDSKDSTYSLSSTLTLSKADYEKHKVYACEVTHQGLSSPVTKSFNRGEC